European Patent Specification EP 3 702 370 B1, published March 26, 2025. Title: Monoclonal Antibody of Human-derived Procalcitonin, and Application Thereof. Applicant: Nanjing Norman Biological Technology Co., Ltd. The sequence listing filed with the application follows.

SEQUENCE LISTING (55 sequences)

SEQ ID NO: 1 - protein, 12 aa, Human
RLLLAALVQDYV

SEQ ID NO: 2 - protein, 116 aa, Human
APFRSALESSPADPATLSEEEARLLLAALVQDYVQMKASELEQEQEREGSSLDSPRSKRCGNLSTCMLGTYTQDFNKFHTFPQTAIGVGAPGKKRDMSSDLERDHRPHVSMPQNAN

SEQ ID NO: 3 - protein, 116 aa, Human
APFRSALESSPADPATLSEDEARLLLAALVQDYVQMKAAELEQEQEREGSSLDSPRSKRCGNLSTCMLGTYTQDFNKFHTFPQTAIGVGAPGKKRDMSSDLERDHRPHVSMPQNAN

SEQ ID NO: 4 - protein, 116 aa, Human
APFRSALESSPADPATLAEDEARLLLAALVQDYVQMKASELEQEQEREGSSLDSPRSKRCGNLSTCMLGTYTQDFNKFHTFPQTAIGVGAPGKKRDMSSDLERDHRPHVSMPQNAN

SEQ ID NO: 5 - DNA, 369 bp, Human
cacggatccgcaccgttccgttctgcgctggaaagctctccagccgatccggccaccctgagcgaagaggaagcgcgtctgctgctggcggcactggtccaggactacgttcagatgaaagcgtctgaactggagcaggaacaggaacgcgaaggtagcagcctggactctccacgttccaagcgctgtggtaacctgagcacttgtatgctgggcacctatactcaggacttcaacaagttccacactttcccgcagactgcgatcggtgtgggcgcaccgggtaagaaacgtgacatgagctccgacctggagcgtgaccaccgtccacatgtatccatgccacagaacgccaactaactcgagcac

SEQ ID NO: 6 - DNA, 369 bp, Human
cacggatccgctccgttccgcagcgcactggagtcctctccagccgaccctgctaccctgtctgaagacgaagcgcgtctgctgctggctgcgctggttcaggactacgtacagatgaaggcggctgaactggaacaagaacaggagcgcgaaggctccagcctggattccccgcgtagcaaacgctgtggcaacctgtccacttgcatgctgggtacctacacccaagactttaacaaatttcacacgtttccgcaaactgctattggcgttggtgccccgggtaagaaacgtgatatgtctagcgacctggaacgcgatcaccgcccgcacgttagcatgccgcagaacgcaaattaactcgagcac

SEQ ID NO: 7 - DNA, 369 bp, Human
cacggatccgcaccatttcgttctgctctggaatcttctcctgctgatcctgcaaccctggctgaagacgaggcgcgtctgctgctggcagcactggttcaggattatgttcagatgaaagcgagcgaactggagcaggaacaggagcgcgagggcagctctctggattctcctcgtagcaaacgttgcggtaacctgagcacctgcatgctgggtacctacacgcaagacttcaacaaattccacacttttccgcagactgcgattggtgtgggtgcgccgggtaaaaagcgtgacatgagctctgacctggaacgtgaccatcgtccgcatgtttctatgccgcagaacgcgaactaactcgagcac

SEQ ID NO: 8 - DNA, 31 bp, Artificial primer
cacggatccgcaccgttccgttctgcgctgg

SEQ ID NO: 9 - DNA, 41 bp, Artificial primer
tggccggatcggctggagagctttccagcgcagaacggaac

SEQ ID NO: 10 - DNA, 41 bp, Artificial primer
cagccgatccggccaccctgagcgaagaggaagcgcgtctg

SEQ ID NO: 11 - DNA, 41 bp, Artificial primer
tcctggaccagtgccgccagcagcagacgcgcttcctcttc

SEQ ID NO: 12 - DNA, 41 bp, Artificial primer
cggcactggtccaggactacgttcagatgaaagcgtctgaa

SEQ ID NO: 13 - DNA, 41 bp, Artificial primer
gttcctgttcctgctccagttcagacgctttcatctgaacg

SEQ ID NO: 14 - DNA, 41 bp, Artificial primer
ctggagcaggaacaggaacgcgaaggtagcagcctggactc

SEQ ID NO: 15 - DNA, 41 bp, Artificial primer
taccacagcgcttggaacgtggagagtccaggctgctacct

SEQ ID NO: 16 - DNA, 41 bp, Artificial primer
gttccaagcgctgtggtaacctgagcacttgtatgctgggc

SEQ ID NO: 17 - DNA, 41 bp, Artificial primer
ttgttgaagtcctgagtataggtgcccagcatacaagtgct

SEQ ID NO: 18 - DNA, 41 bp, Artificial primer
acctatactcaggacttcaacaagttccacactttcccgca

SEQ ID NO: 19 - DNA, 41 bp, Artificial primer
gtgcgcccacaccgatcgcagtctgcgggaaagtgtggaac

SEQ ID NO: 20 - DNA, 41 bp, Artificial primer
tcggtgtgggcgcaccgggtaagaaacgtgacatgagctcc

SEQ ID NO: 21 - DNA, 41 bp, Artificial primer
cggtggtcacgctccaggtcggagctcatgtcacgtttctt

SEQ ID NO: 22 - DNA, 41 bp, Artificial primer
tggagcgtgaccaccgtccacatgtatccatgccacagaac

SEQ ID NO: 23 - DNA, 39 bp, Artificial primer
gtgctcgagttagttggcgttctgtggcatggatacatg

SEQ ID NO: 24 - DNA, 30 bp, Artificial primer
cacggatccgctccgttccgcagcgcactg

SEQ ID NO: 25 - DNA, 41 bp, Artificial primer
tagcagggtcggctggagaggactccagtgcgctgcggaac

SEQ ID NO: 26 - DNA, 41 bp, Artificial primer
ccagccgaccctgctaccctgtctgaagacgaagcgcgtct

SEQ ID NO: 27 - DNA, 41 bp, Artificial primer
cctgaaccagcgcagccagcagcagacgcgcttcgtcttca

SEQ ID NO: 28 - DNA, 41 bp, Artificial primer
gctgcgctggttcaggactacgtacagatgaaggcggctga

SEQ ID NO: 29 - DNA, 41 bp, Artificial primer
cgcgctcctgttcttgttccagttcagccgccttcatctgt

SEQ ID NO: 30 - DNA, 41 bp, Artificial primer
aacaagaacaggagcgcgaaggctccagcctggattccccg

SEQ ID NO: 31 - DNA, 41 bp, Artificial primer
caggttgccacagcgtttgctacgcggggaatccaggctgg

SEQ ID NO: 32 - DNA, 41 bp, Artificial primerÎï
aacgctgtggcaacctgtccacttgcatgctgggtacctac

SEQ ID NO: 33 - DNA, 44 bp, Artificial primer
gtgaaatttgttaaagtcttgggtgtaggtacccagcatgcaag

SEQ ID NO: 34 - DNA, 43 bp, Artificial primer
acccaagactttaacaaatttcacacgtttccgcaaactgcta

SEQ ID NO: 35 - DNA, 41 bp, Artificial primer
ttacccggggcaccaacgccaatagcagtttgcggaaacgt

SEQ ID NO: 36 - DNA, 41 bp, Artificial primer
gttggtgccccgggtaagaaacgtgatatgtctagcgacct

SEQ ID NO: 37 - DNA, 41 bp, Artificial primer
gcgggcggtgatcgcgttccaggtcgctagacatatcacgt

SEQ ID NO: 38 - DNA, 41 bp, Artificial primer
gcgatcaccgcccgcacgttagcatgccgcagaacgcaaat

SEQ ID NO: 39 - DNA, 29 bp, Artificial primer
gtgctcgagttaatttgcgttctgcggca

SEQ ID NO: 40 - DNA, 36 bp, Artificial primer
cacggatccgcaccatttcgttctgctctggaatct

SEQ ID NO: 41 - DNA, 41 bp, Artificial primer
gttgcaggatcagcaggagaagattccagagcagaacgaaa

SEQ ID NO: 42 - DNA, 41 bp, Artificial primer
ctcctgctgatcctgcaaccctggctgaagacgaggcgcgt

SEQ ID NO: 43 - DNA, 41 bp, Artificial primer
cctgaaccagtgctgccagcagcagacgcgcctcgtcttca

SEQ ID NO: 44 - DNA, 41 bp, Artificial primer
ggcagcactggttcaggattatgttcagatgaaagcgagcg

SEQ ID NO: 45 - DNA, 41 bp, Artificial primer
gctcctgttcctgctccagttcgctcgctttcatctgaaca

SEQ ID NO: 46 - DNA, 41 bp, Artificial primer
tggagcaggaacaggagcgcgagggcagctctctggattct

SEQ ID NO: 47 - DNA, 41 bp, Artificial primer
taccgcaacgtttgctacgaggagaatccagagagctgccc

SEQ ID NO: 48 - DNA, 41 bp, Artificial primer
cgtagcaaacgttgcggtaacctgagcacctgcatgctggg

SEQ ID NO: 49 - DNA, 41 bp, Artificial primer
tttgttgaagtcttgcgtgtaggtacccagcatgcaggtgc

SEQ ID NO: 50 - DNA, 42 bp, Artificial primer
ctacacgcaagacttcaacaaattccacacttttccgcagac

SEQ ID NO: 51 - DNA, 41 bp, Artificial primer
ggcgcacccacaccaatcgcagtctgcggaaaagtgtggaa

SEQ ID NO: 52 - DNA, 41 bp, Artificial primer
tggtgtgggtgcgccgggtaaaaagcgtgacatgagctctg

SEQ ID NO: 53 - DNA, 41 bp, Artificial primer
ggacgatggtcacgttccaggtcagagctcatgtcacgctt

SEQ ID NO: 54 - DNA, 41 bp, Artificial primer
ggaacgtgaccatcgtccgcatgtttctatgccgcagaacg

SEQ ID NO: 55 - DNA, 37 bp, Artificial primer
gtgctcgagttagttcgcgttctgcggcatagaaaca